European Patent Application EP 4 477 232 A1, published December 18, 2024. Title: RECOMBINANT MULTIVALENT VACCINE. Applicant: SHANGHAI PUBLIC HEALTH CLINICAL CENTER. The sequence listing filed with the application follows.

SEQUENCE LISTING (22 sequences)

SEQ ID NO: 1 - protein, 171 aa, synthetic construct
MAQVINTNSLSLITQNNINKNQSALSSSIERASSGAAAGSAKDDAAGQAIANRFTSNIKGLGSAARGAGAGISAAGTTEGALSGANNNLQRVRELTVQATTGTNSESDLSSIQDEIKSRLDEISAASGGGSAGGAGALAKNGSAAISAGASASSTITADAASIAAGALGLG

SEQ ID NO: 2 - DNA, 513 bp, synthetic construct
  source 1..513: mol_type = other DNA
atggcccaagtgatcaacaccaacagcctgagcctgatcacccagaacaatatcaacaagaaccagagcgctctgtccagcagcatcgagagagcctctagcggcgctgctgccggctctgcaaaggacgatgccgccggccaggccatcgctaatagatttaccagcaacatcaagggcctgggatctgccgctagaggcgccggagcaggaatctccgccgccggaaccacagaaggagcactgagcggcgccaacaacaacctgcaaagagtgcgggaactgaccgtgcaggccaccaccggaacaaacagcgagagcgacctgagcagcatccaggacgaaatcaagtcaaggctggatgagatcagcgccgcctctggcggaggcagcgcaggcggggctggcgccctggccaaaaacggctcagccgccatctccgccggagctagcgctagcagcaccatcacagccgatgctgccagcatcgccgccggcgccctgggcctgggc

SEQ ID NO: 3 - protein, 94 aa, synthetic construct
ATTTDPLKALDDAIASVAKFASSLGAASGALSSAATNLSSTTTALSGASSAIGDADSATGVSGASAAQAASSAGGSVLAKANQVASSVLSAASG

SEQ ID NO: 4 - DNA, 282 bp, synthetic construct
  source 1..282: mol_type = other DNA
gcaaccaccacggatccgctgaaggccctggacgacgccattgcgagtgttgccaaattcgccagcagtctgggcgccgcctctggcgctctgagcagcgccgctacaaacctgagctctacaacaacagccctctctggcgcttcctccgccatcggcgacgccgatagcgccaccggcgtctctggcgccagcgccgctcaggccgcctcttctgcgggtggcagcgtgctggctaaagccaaccaggtggccagcagcgtgctctccgctgcctctgga

SEQ ID NO: 5 - protein, 209 aa, SARS-CoV-2 Delta variant
RVQPTESIVRFPNITNLCPFGEVFNATRFASVYAWNRKRISNCVADYSVLYNSASFSTFKCYGVSPTKLNDLCFTNVYADSFVIRGDEVRQIAPGQTGKIADYNYKLPDDFTGCVIAWNSNNLDSKVGGNYNYRYRLFRKSNLKPFERDISTEIYQAGSKPCNGVEGFNCYFPLQSYGFQPTNGVGYQPYRVVVLSFELLHAPATVCGP

SEQ ID NO: 6 - DNA, 627 bp, SARS-CoV-2 Delta variant
  source 1..627: mol_type = other DNA
agagtgcagccaaccgaaagcatcgttagattcccaaacatcaccaacctctgtcctttcggcgaggtgttcaacgccacgagattcgcctccgtgtacgcctggaaccggaagcggatcagcaattgcgtggccgactacagcgtgctgtacaatagcgcctctttcagcacttttaagtgctacggcgtgtcccctacaaagctgaacgacctgtgcttcacaaatgtgtacgccgacagcttcgtgattagaggcgatgaggtgcggcagatcgcccctggacaaacaggcaagatcgccgattacaactataagctgcctgacgacttcaccggctgtgtgatcgcttggaacagcaacaacctggatagcaaggtcggcggaaattacaactaccggtatagactgttcagaaagagcaacctgaaaccttttgagcgcgacatcagcaccgagatctaccaggccggcagcaagccttgcaacggcgtggaaggctttaactgctacttccccctgcagagctacggcttccagcctaccaatggcgtgggctaccagccctaccgggtcgtggtgctgagcttcgagctgctgcacgcccctgccaccgtgtgcggcccc

SEQ ID NO: 7 - protein, 209 aa, SARS-CoV-2 Omicron variant
RVQPTESIVRFPNITNLCPFDEVFNATRFASVYAWNRKRISNCVADYSVLYNLAPFFTFKCYGVSPTKLNDLCFTNVYADSFVIRGDEVRQIAPGQTGNIADYNYKLPDDFTGCVIAWNSNKLDSKVSGNYNYLYRLFRKSNLKPFERDISTEIYQAGNKPCNGVAGFNCYFPLRSYSFRPTYGVGHQPYRVVVLSFELLHAPATVCGP

SEQ ID NO: 8 - DNA, 627 bp, SARS-CoV-2 Omicron variant
  source 1..627: mol_type = other DNA
cgggtgcagcctaccgagtcgatcgtgcggttcccgaacattacaaacctgtgccccttcgacgaggtgtttaacgccacccgcttcgccagcgtgtacgcctggaacagaaagagaatcagcaactgcgtagctgattactccgtgctgtacaacctggccccatttttcaccttcaagtgctacggagtgagcccaaccaagctgaatgacctttgtttcactaacgtgtacgctgactccttcgtgatcagaggcgacgaagtgcggcagatcgcacctggccagacaggcaacatcgccgactacaactacaaactgccagatgacttcaccggctgtgtgatcgcgtggaatagtaacaagctggattccaaagtgtccggaaactataactacctgtaccgactgttccggaagagcaatctgaagcccttcgagagagacatcagcaccgaaatctaccaggccggaaataaaccttgtaacggcgttgctggatttaactgctactttcctctgaggagctacagctttagacccacatacggcgttggccaccagccctaccgggtggtggtgctgagcttcgaactgctgcatgcccctgctacagtgtgcggccct

SEQ ID NO: 9 - protein, 209 aa, SARS-CoV-2 original strain
RVQPTESIVRFPNITNLCPFGEVFNATRFASVYAWNRKRISNCVADYSVLYNSASFSTFKCYGVSPTKLNDLCFTNVYADSFVIRGDEVRQIAPGQTGKIADYNYKLPDDFTGCVIAWNSNNLDSKVGGNYNYLYRLFRKSNLKPFERDISTEIYQAGSTPCNGVEGFNCYFPLQSYGFQPTNGVGYQPYRVVVLSFELLHAPATVCGP

SEQ ID NO: 10 - DNA, 627 bp, SARS-CoV-2 original strain
  source 1..627: mol_type = other DNA
agagtgcagccaaccgaaagcatcgttagattcccaaacatcaccaacctctgtcctttcggcgaggtgttcaacgccacgagattcgcctccgtgtacgcctggaaccggaagcggatcagcaattgcgtggccgactacagcgtgctgtacaatagcgcctctttcagcacttttaagtgctacggcgtgtcccctacaaagctgaacgacctgtgcttcacaaatgtgtacgccgacagcttcgtgattagaggcgatgaggtgcggcagatcgcccctggacaaacaggcaagatcgccgattacaactataagctgcctgacgacttcaccggctgtgtgatcgcttggaacagcaacaacctggatagcaaggtcggcggaaattacaactacctgtatagactgttcagaaagagcaacctgaaaccttttgagcgcgacatcagcaccgagatctaccaggccggcagcaccccttgcaacggcgtggaaggctttaactgctacttccccctgcagagctacggcttccagcctaccaatggcgtgggctaccagccctaccgggtcgtggtgctgagcttcgagctgctgcacgcccctgccaccgtgtgcggcccc

SEQ ID NO: 11 - protein, 209 aa, SARS-CoV-2 Gamma variant
RVQPTESIVRFPNITNLCPFGEVFNATRFASVYAWNRKRISNCVADYSVLYNSASFSTFKCYGVSPTKLNDLCFTNVYADSFVIRGDEVRQIAPGQTGTIADYNYKLPDDFTGCVIAWNSNNLDSKVGGNYNYLYRLFRKSNLKPFERDISTEIYQAGSTPCNGVKGFNCYFPLQSYGFQPTYGVGYQPYRVVVLSFELLHAPATVCGP

SEQ ID NO: 12 - DNA, 627 bp, SARS-CoV-2 Gamma variant
  source 1..627: mol_type = other DNA
agagtgcagccaaccgaaagcatcgttagattcccaaacatcaccaacctctgtcctttcggcgaggtgttcaacgccacgagattcgcctccgtgtacgcctggaaccggaagcggatcagcaattgcgtggccgactacagcgtgctgtacaatagcgcctctttcagcacttttaagtgctacggcgtgtcccctacaaagctgaacgacctgtgcttcacaaatgtgtacgccgacagcttcgtgattagaggcgatgaggtgcggcagatcgcccctggacaaacaggcaccatcgccgattacaactataagctgcctgacgacttcaccggctgtgtgatcgcttggaacagcaacaacctggatagcaaggtcggcggaaattacaactacctgtatagactgttcagaaagagcaacctgaaaccttttgagcgcgacatcagcaccgagatctaccaggccggcagcaccccttgcaacggcgtgaagggctttaactgctacttccccctgcagagctacggcttccagcctacctatggcgtgggctaccagccctaccgggtcgtggtgctgagcttcgagctgctgcacgcccctgccaccgtgtgcggcccc

SEQ ID NO: 13 - protein, 208 aa, SARS-CoV-2 SHC014 variant
RVAPSKEVVRFPNITNLCPFGEVFNATTFPSVYAWERKRISNCVADYSVLYNSTSFSTFKCYGVSATKLNDLCFSNVYADSFVVKGDDVRQIAPGQTGVIADYNYKLPDDFLGCVLAWNTNSKDSSTSGNYNYLYRWVRRSKLNPYERDLSNDIYSPGGQSCSAVGPNCYNPLRPYGFFTTAGVGHQPYRVVVLSFELLNAPATVCGP

SEQ ID NO: 14 - DNA, 624 bp, SARS-CoV-2 SHC014 variant
  source 1..624: mol_type = other DNA
agagtggcccctagcaaggaggtggtgcggttcccaaacatcactaacctgtgccccttcggagaggtgtttaacgctaccactttccctagcgtgtacgcctgggagagaaagaggattagcaactgcgtggccgactattccgtgctgtacaactccaccagcttctccacctttaagtgctacggcgtgagcgctaccaagttgaacgacctgtgcttcagcaacgtctacgctgacagcttcgtggtcaaaggagacgacgtgagacaaatcgcccctggacaaacaggagtgatcgctgattacaactacaagctgccagatgactttctgggctgcgtcctggcttggaacaccaactccaaagatagcagcacctccggaaactacaactatctgtacaggtgggtgcgcaggtccaaactcaacccctacgagcgcgatctgtcaaacgacatttacagccctggaggccagtcatgctccgctgtgggacctaactgttacaaccctctgcgcccatatggattcttcaccaccgccggagtgggacatcaaccttatagagtggtcgtcctgtctttcgagttgttgaacgctcctgccacagtctgtggacct

SEQ ID NO: 15 - protein, 208 aa, SARS-CoV-2 WIV1 variant
RVAPSKEVVRFPNITNLCPFGEVFNATTFPSVYAWERKRISNCVADYSVLYNSTSFSTFKCYGVSATKLNDLCFSNVYADSFVVKGDDVRQIAPGQTGVIADYNYKLPDDFTGCVLAWNTRNIDATQTGNYNYKYRSLRHGKLRPFERDISNVPFSPDGKPCTPPAFNCYWPLNDYGFYITNGIGYQPYRVVVLSFELLNAPATVCGP

SEQ ID NO: 16 - DNA, 624 bp, SARS-CoV-2 WIV1 variant
  source 1..624: mol_type = other DNA
agagtggcccctagcaaggaggtggtgcggttcccaaacattaccaacctgtgccctttcggcgaagtcttcaatgctactaccttcccttccgtgtacgcctgggaaaggaagagaatttccaactgcgtggccgactattccgtgctgtacaactccaccagcttctccacctttaagtgctacggcgtgagcgctaccaagctcaacgacctgtgctttagcaacgtctacgccgactcctttgtggtcaagggagacgacgtgagacagatcgctcctggacaaaccggagtgattgctgactacaactacaaactgccagatgacttcaccggctgcgtcttggcttggaacaccagaaacatcgacgctacccaaaccggcaactataactacaagtacaggagcctcaggcacggaaagctgaggccttttgagcgcgacatcagcaatgtgccttttagccccgacggaaaaccttgcaccccacccgcctttaattgctactggccattgaacgactacggattttacatcactaacggcattggctatcagccttacagggtggtcgtcctgtcctttgagctgctcaatgcccctgctactgtgtgcggacca

SEQ ID NO: 17 - protein, 902 aa, synthetic construct
RVQPTESIVRFPNITNLCPFDEVFNATRFASVYAWNRKRISNCVADYSVLYNLAPFFTFKCYGVSPTKLNDLCFTNVYADSFVIRGDEVRQIAPGQTGNIADYNYKLPDDFTGCVIAWNSNKLDSKVSGNYNYLYRLFRKSNLKPFERDISTEIYQAGNKPCNGVAGFNCYFPLRSYSFRPTYGVGHQPYRVVVLSFELLHAPATVCGPMAQVINTNSLSLITQNNINKNQSALSSSIERASSGAAAGSAKDDAAGQAIANRFTSNIKGLGSAARGAGAGISAAGTTEGALSGANNNLQRVRELTVQATTGTNSESDLSSIQDEIKSRLDEISAASGGGSAGGAGALAKNGSAAISAGASASSTITADAASIAAGALGLGASGGGSRVQPTESIVRFPNITNLCPFGEVFNATRFASVYAWNRKRISNCVADYSVLYNSASFSTFKCYGVSPTKLNDLCFTNVYADSFVIRGDEVRQIAPGQTGKIADYNYKLPDDFTGCVIAWNSNNLDSKVGGNYNYRYRLFRKSNLKPFERDISTEIYQAGSKPCNGVEGFNCYFPLQSYGFQPTNGVGYQPYRVVVLSFELLHAPATVCGPGGGSATTTDPLKALDDAIASVAKFASSLGAASGALSSAATNLSSTTTALSGASSAIGDADSATGVSGASAAQAASSAGGSVLAKANQVASSVLSAASGRVQPTESIVRFPNITNLCPFDEVFNATRFASVYAWNRKRISNCVADYSVLYNLAPFFTFKCYGVSPTKLNDLCFTNVYADSFVIRGDEVRQIAPGQTGNIADYNYKLPDDFTGCVIAWNSNKLDSKVSGNYNYLYRLFRKSNLKPFERDISTEIYQAGNKPCNGVAGFNCYFPLRSYSFRPTYGVGHQPYRVVVLSFELLHAPATVCGP

SEQ ID NO: 18 - DNA, 2706 bp, synthetic construct
  source 1..2706: mol_type = other DNA
cgggtgcagcctaccgagtcgatcgtgcggttcccgaacattacaaacctgtgccccttcgacgaggtgtttaacgccacccgcttcgccagcgtgtacgcctggaacagaaagagaatcagcaactgcgtagctgattactccgtgctgtacaacctggccccatttttcaccttcaagtgctacggagtgagcccaaccaagctgaatgacctttgtttcactaacgtgtacgctgactccttcgtgatcagaggcgacgaagtgcggcagatcgcacctggccagacaggcaacatcgccgactacaactacaaactgccagatgacttcaccggctgtgtgatcgcgtggaatagtaacaagctggattccaaagtgtccggaaactataactacctgtaccgactgttccggaagagcaatctgaagcccttcgagagagacatcagcaccgaaatctaccaggccggaaataaaccttgtaacggcgttgctggatttaactgctactttcctctgaggagctacagctttagacccacatacggcgttggccaccagccctaccgggtggtggtgctgagcttcgaactgctgcatgcccctgctacagtgtgcggccctatggcccaagtgatcaacaccaacagcctgagcctgatcacccagaacaatatcaacaagaaccagagcgctctgtccagcagcatcgagagagcctctagcggcgctgctgccggctctgcaaaggacgatgccgccggccaggccatcgctaatagatttaccagcaacatcaagggcctgggatctgccgctagaggcgccggagcaggaatctccgccgccggaaccacagaaggagcactgagcggcgccaacaacaacctgcaaagagtgcgggaactgaccgtgcaggccaccaccggaacaaacagcgagagcgacctgagcagcatccaggacgaaatcaagtcaaggctggatgagatcagcgccgcctctggcggaggcagcgcaggcggggctggcgccctggccaaaaacggctcagccgccatctccgccggagctagcgctagcagcaccatcacagccgatgctgccagcatcgccgccggcgccctgggcctgggcgctagcggcggaggttctagagtgcagccaaccgaaagcatcgttagattcccaaacatcaccaacctctgtcctttcggcgaggtgttcaacgccacgagattcgcctccgtgtacgcctggaaccggaagcggatcagcaattgcgtggccgactacagcgtgctgtacaatagcgcctctttcagcacttttaagtgctacggcgtgtcccctacaaagctgaacgacctgtgcttcacaaatgtgtacgccgacagcttcgtgattagaggcgatgaggtgcggcagatcgcccctggacaaacaggcaagatcgccgattacaactataagctgcctgacgacttcaccggctgtgtgatcgcttggaacagcaacaacctggatagcaaggtcggcggaaattacaactaccggtatagactgttcagaaagagcaacctgaaaccttttgagcgcgacatcagcaccgagatctaccaggccggcagcaagccttgcaacggcgtggaaggctttaactgctacttccccctgcagagctacggcttccagcctaccaatggcgtgggctaccagccctaccgggtcgtggtgctgagcttcgagctgctgcacgcccctgccaccgtgtgcggccccggcggcggctctgcaaccaccacggatccgctgaaggccctggacgacgccattgcgagtgttgccaaattcgccagcagtctgggcgccgcctctggcgctctgagcagcgccgctacaaacctgagctctacaacaacagccctctctggcgcttcctccgccatcggcgacgccgatagcgccaccggcgtctctggcgccagcgccgctcaggccgcctcttctgcgggtggcagcgtgctggctaaagccaaccaggtggccagcagcgtgctctccgctgcctctggacgggtgcagcctaccgagtcgatcgtgcggttcccgaacattacaaacctgtgccccttcgacgaggtgtttaacgccacccgcttcgccagcgtgtacgcctggaacagaaagagaatcagcaactgcgtagctgattactccgtgctgtacaacctggccccatttttcaccttcaagtgctacggagtgagcccaaccaagctgaatgacctttgtttcactaacgtgtacgctgactccttcgtgatcagaggcgacgaagtgcggcagatcgcacctggccagacaggcaacatcgccgactacaactacaaactgccagatgacttcaccggctgtgtgatcgcgtggaatagtaacaagctggattccaaagtgtccggaaactataactacctgtaccgactgttccggaagagcaatctgaagcccttcgagagagacatcagcaccgaaatctaccaggccggaaataaaccttgtaacggcgttgctggatttaactgctactttcctctgaggagctacagctttagacccacatacggcgttggccaccagccctaccgggtggtggtgctgagcttcgaactgctgcatgcccctgctacagtgtgcggccct

SEQ ID NO: 19 - protein, 900 aa, synthetic construct
RVQPTESIVRFPNITNLCPFDEVFNATRFASVYAWNRKRISNCVADYSVLYNLAPFFTFKCYGVSPTKLNDLCFTNVYADSFVIRGDEVRQIAPGQTGNIADYNYKLPDDFTGCVIAWNSNKLDSKVSGNYNYLYRLFRKSNLKPFERDISTEIYQAGNKPCNGVAGFNCYFPLRSYSFRPTYGVGHQPYRVVVLSFELLHAPATVCGPMAQVINTNSLSLITQNNINKNQSALSSSIERASSGAAAGSAKDDAAGQAIANRFTSNIKGLGSAARGAGAGISAAGTTEGALSGANNNLQRVRELTVQATTGTNSESDLSSIQDEIKSRLDEISAASGGGSAGGAGALAKNGSAAISAGASASSTITADAASIAAGALGLGASGGGSRVAPSKEVVRFPNITNLCPFGEVFNATTFPSVYAWERKRISNCVADYSVLYNSTSFSTFKCYGVSATKLNDLCFSNVYADSFVVKGDDVRQIAPGQTGVIADYNYKLPDDFLGCVLAWNTNSKDSSTSGNYNYLYRWVRRSKLNPYERDLSNDIYSPGGQSCSAVGPNCYNPLRPYGFFTTAGVGHQPYRVVVLSFELLNAPATVCGPGGGSATTTDPLKALDDAIASVAKFASSLGAASGALSSAATNLSSTTTALSGASSAIGDADSATGVSGASAAQAASSAGGSVLAKANQVASSVLSAASGRVAPSKEVVRFPNITNLCPFGEVFNATTFPSVYAWERKRISNCVADYSVLYNSTSFSTFKCYGVSATKLNDLCFSNVYADSFVVKGDDVRQIAPGQTGVIADYNYKLPDDFTGCVLAWNTRNIDATQTGNYNYKYRSLRHGKLRPFERDISNVPFSPDGKPCTPPAFNCYWPLNDYGFYITNGIGYQPYRVVVLSFELLNAPATVCGP

SEQ ID NO: 20 - DNA, 2700 bp, synthetic construct
  source 1..2700: mol_type = other DNA
cgggtgcagcctaccgagtcgatcgtgcggttcccgaacattacaaacctgtgccccttcgacgaggtgtttaacgccacccgcttcgccagcgtgtacgcctggaacagaaagagaatcagcaactgcgtagctgattactccgtgctgtacaacctggccccatttttcaccttcaagtgctacggagtgagcccaaccaagctgaatgacctttgtttcactaacgtgtacgctgactccttcgtgatcagaggcgacgaagtgcggcagatcgcacctggccagacaggcaacatcgccgactacaactacaaactgccagatgacttcaccggctgtgtgatcgcgtggaatagtaacaagctggattccaaagtgtccggaaactataactacctgtaccgactgttccggaagagcaatctgaagcccttcgagagagacatcagcaccgaaatctaccaggccggaaataaaccttgtaacggcgttgctggatttaactgctactttcctctgaggagctacagctttagacccacatacggcgttggccaccagccctaccgggtggtggtgctgagcttcgaactgctgcatgcccctgctacagtgtgcggccctatggcccaagtgatcaacaccaacagcctgagcctgatcacccagaacaatatcaacaagaaccagagcgctctgtccagcagcatcgagagagcctctagcggcgctgctgccggctctgcaaaggacgatgccgccggccaggccatcgctaatagatttaccagcaacatcaagggcctgggatctgccgctagaggcgccggagcaggaatctccgccgccggaaccacagaaggagcactgagcggcgccaacaacaacctgcaaagagtgcgggaactgaccgtgcaggccaccaccggaacaaacagcgagagcgacctgagcagcatccaggacgaaatcaagtcaaggctggatgagatcagcgccgcctctggcggaggcagcgcaggcggggctggcgccctggccaaaaacggctcagccgccatctccgccggagctagcgctagcagcaccatcacagccgatgctgccagcatcgccgccggcgccctgggcctgggcgctagcggcggaggttctagagtggcccctagcaaggaggtggtgcggttcccaaacatcactaacctgtgccccttcggagaggtgtttaacgctaccactttccctagcgtgtacgcctgggagagaaagaggattagcaactgcgtggccgactattccgtgctgtacaactccaccagcttctccacctttaagtgctacggcgtgagcgctaccaagttgaacgacctgtgcttcagcaacgtctacgctgacagcttcgtggtcaaaggagacgacgtgagacaaatcgcccctggacaaacaggagtgatcgctgattacaactacaagctgccagatgactttctgggctgcgtcctggcttggaacaccaactccaaagatagcagcacctccggaaactacaactatctgtacaggtgggtgcgcaggtccaaactcaacccctacgagcgcgatctgtcaaacgacatttacagccctggaggccagtcatgctccgctgtgggacctaactgttacaaccctctgcgcccatatggattcttcaccaccgccggagtgggacatcaaccttatagagtggtcgtcctgtctttcgagttgttgaacgctcctgccacagtctgtggacctggcggcggctctgcaaccaccacggatccgctgaaggccctggacgacgccattgcgagtgttgccaaattcgccagcagtctgggcgccgcctctggcgctctgagcagcgccgctacaaacctgagctctacaacaacagccctctctggcgcttcctccgccatcggcgacgccgatagcgccaccggcgtctctggcgccagcgccgctcaggccgcctcttctgcgggtggcagcgtgctggctaaagccaaccaggtggccagcagcgtgctctccgctgcctctggaagagtggcccctagcaaggaggtggtgcggttcccaaacatcactaacctgtgccccttcggagaggtgtttaacgctaccactttccctagcgtgtacgcctgggagagaaagaggattagcaactgcgtggccgactattccgtgctgtacaactccaccagcttctccacctttaagtgctacggcgtgagcgctaccaagttgaacgacctgtgcttcagcaacgtctacgctgacagcttcgtggtcaaaggagacgacgtgagacaaatcgcccctggacaaacaggagtgatcgctgattacaactacaagctgccagatgactttctgggctgcgtcctggcttggaacaccaactccaaagatagcagcacctccggaaactacaactatctgtacaggtgggtgcgcaggtccaaactcaacccctacgagcgcgatctgtcaaacgacatttacagccctggaggccagtcatgctccgctgtgggacctaactgttacaaccctctgcgcccatatggattcttcaccaccgccggagtgggacatcaaccttatagagtggtcgtcctgtctttcgagttgttgaacgctcctgccacagtctgtggacct

SEQ ID NO: 21 - protein, 267 aa, synthetic construct
MAQVINTNSLSLITQNNINKNQSALSSSIERLSSGLRINSAKDDAAGQAIANRFTSNIKGLTQAARNANDGISVAQTTEGALSEINNNLQRVRELTVQATTGTNSESDLSSIQDEIKSRLDEIDRVSGQTQFNGVNVLAKNGSMKIQVGANDNQTITIDLKQIDAKTLGLDASATTTDPLKALDDAIASVDKFRSSLGAVQNRLDSAVTNLNNTTTNLSEAQSRIQDADYATEVSNMSKAQIIQQAGNSVLAKANQVPQQVLSLLQG

SEQ ID NO: 22 - DNA, 801 bp, synthetic construct
  source 1..801: mol_type = other DNA
atggcacaagtcattaataccaacagcctctcgctgatcactcaaaataatatcaacaagaaccagtctgcgctgtcgagttctatcgagcgtctgtcttctggcttgcgtattaacagcgcgaaggatgacgcagcgggtcaggcgattgctaaccgtttcacctctaacattaaaggcctgactcaggcggcccgtaacgccaacgacggtatctccgttgcgcagaccaccgaaggcgcgctgtccgaaatcaacaacaacttacagcgtgtgcgtgaactgacggtacaggccactaccggtactaactctgagtctgatctgtcttctatccaggacgaaattaaatcccgtctggatgaaattgaccgcgtatctggtcagacccagttcaacggcgtgaacgtgctggcaaaaaatggctccatgaaaatccaggttggcgcaaatgataaccagactatcactatcgatctgaagcagattgatgctaaaactcttggccttgatgctagcgctacgacgacggatccgctgaaagcgctggacgatgctatcgcatctgtagacaaattccgttcttccctcggtgcggtgcaaaaccgtctggattccgcggttaccaacctgaacaacaccactaccaacctgtctgaagcgcagtcccgtattcaggacgccgactatgcgaccgaagtgtccaatatgtcgaaagcgcagatcatccagcaggccggtaactccgtgttggcaaaagctaaccaggtaccgcagcaggttctgtctctgctgcagggt